European Patent Application EP 4 119 163 A1, published January 18, 2023. Title: Therapeutic agent for virus infection. Applicant: The University of Tokyo. The sequence listing filed with the application follows.

SEQUENCE LISTING (8 sequences)

SEQ ID NO: 1 - DNA, 20 bp, Artificial Sequence
  Synthetic nucleic acid
gctttcacggaggttcgacg

SEQ ID NO: 2 - DNA, 20 bp, Artificial Sequence
  Synthetic nucleic acid
atgttgcagttcggctcgat

SEQ ID NO: 3 - DNA, 20 bp, Artificial Sequence
  Synthetic nucleic acid
atgagcaccatctacagtac

SEQ ID NO: 4 - DNA, 20 bp, Artificial Sequence
  Synthetic nucleic acid
tgctgctcagtccaccattg

SEQ ID NO: 5 - DNA, 20 bp, Artificial Sequence
  Synthetic nucleic acid
aaattttggggaccaggaac

SEQ ID NO: 6 - DNA, 20 bp, Artificial Sequence
  Synthetic nucleic acid
tggcagctgtgtaggtcaac

SEQ ID NO: 7 - DNA, 20 bp, Artificial Sequence
  Synthetic nucleic acid
gcaccgtcaaggctgagaac

SEQ ID NO: 8 - DNA, 19 bp, Artificial Sequence
  Synthetic nucleic acid
tggtgaagacgccagtgga